European Patent Application EP 4 582 437 A1, published July 9, 2025. Title: 环肽及其制备方法、包括其的复合物、及其用途. Applicant: 核欣（苏州）医药科技有限公司. Application CN. The sequence listing filed with the application follows.

SEQUENCE LISTING (30 sequences)

SEQ ID NO: 1 - protein, 5 aa, synthetic construct
  REGION 1..5: note = circular
NGRDK

SEQ ID NO: 2 - protein, 5 aa, synthetic construct
  REGION 1..5: note = circular
NGRYK

SEQ ID NO: 3 - protein, 5 aa, synthetic construct
  REGION 1..5: note = circular
NGRTK

SEQ ID NO: 4 - protein, 5 aa, synthetic construct
  REGION 1..5: note = circular
NGRFK

SEQ ID NO: 5 - protein, 6 aa, synthetic construct
  REGION 1..6: note = circular
NGRTKE

SEQ ID NO: 6 - protein, 6 aa, synthetic construct
  REGION 1..6: note = circular
NGRTKV

SEQ ID NO: 7 - protein, 6 aa, synthetic construct
  REGION 1..6: note = circular
NGRTKF

SEQ ID NO: 8 - protein, 6 aa, synthetic construct
  REGION 1..6: note = circular
NGRTKG

SEQ ID NO: 9 - protein, 6 aa, synthetic construct
  REGION 1..6: note = circular
NGRTKY

SEQ ID NO: 10 - protein, 6 aa, synthetic construct
  REGION 1..6: note = circular
NGRTCE

SEQ ID NO: 11 - protein, 6 aa, synthetic construct
  REGION 1..6: note = circular
NGRTCV

SEQ ID NO: 12 - protein, 6 aa, synthetic construct
  REGION 1..6: note = circular
NGRTCF

SEQ ID NO: 13 - protein, 6 aa, synthetic construct
  REGION 1..6: note = circular
NGRTCG

SEQ ID NO: 14 - protein, 6 aa, synthetic construct
  REGION 1..6: note = circular
NGRTCY

SEQ ID NO: 15 - protein, 6 aa, synthetic construct
  SITE 6: note = D-tyrosine
  REGION 1..6: note = circular
NGRTKY

SEQ ID NO: 16 - protein, 6 aa, synthetic construct
  SITE 6: note = D-valine
  REGION 1..6: note = circular
NGRTKV

SEQ ID NO: 17 - protein, 6 aa, synthetic construct
  SITE 6: note = D-phenylalanine
  REGION 1..6: note = circular
NGRTKF

SEQ ID NO: 18 - protein, 6 aa, synthetic construct
  SITE 4: note = D-threonine
  REGION 1..6: note = circular
NGRTKY

SEQ ID NO: 19 - protein, 6 aa, synthetic construct
  SITE 5: note = D-lysine
  REGION 1..6: note = circular
NGRTKY

SEQ ID NO: 20 - protein, 6 aa, synthetic construct
  SITE 1: note = N-methyl-L-asparagine
  REGION 1..6: note = circular
XGRTKY

SEQ ID NO: 21 - protein, 6 aa, synthetic construct
  SITE 2: note = MeGly
  REGION 1..6: note = circular
NXRTKY

SEQ ID NO: 22 - protein, 6 aa, synthetic construct
  SITE 2: note = MeGly
  SITE 6: note = D-tyrosine
  REGION 1..6: note = circular
NXRTKY

SEQ ID NO: 23 - protein, 6 aa, synthetic construct
  SITE 2: note = MeGly
  SITE 5: note = Orn
  REGION 1..6: note = circular
NXRTXY

SEQ ID NO: 24 - protein, 6 aa, synthetic construct
  SITE 2: note = MeGly
  SITE 5: note = Dbu
  REGION 1..6: note = circular
NXRTXY

SEQ ID NO: 25 - protein, 6 aa, synthetic construct
  SITE 2: note = MeGly
  SITE 5: note = D-cysteine
  REGION 1..6: note = circular
NXRTCY

SEQ ID NO: 26 - protein, 6 aa, synthetic construct
  SITE 1: note = N-methyl-L-asparagine
  SITE 5: note = Dbu
  REGION 1..6: note = circular
XGRTXY

SEQ ID NO: 27 - protein, 6 aa, synthetic construct
  SITE 1: note = N-methyl-L-asparagine
  SITE 5: note = Orn
  REGION 1..6: note = circular
XGRTXY

SEQ ID NO: 28 - protein, 6 aa, synthetic construct
  SITE 1: note = N-methyl-L-asparagine
  SITE 5: note = L-cysteine
  REGION 1..6: note = circular
XGRTCY

SEQ ID NO: 29 - protein, 5 aa, synthetic construct
  REGION 1..5: note = circular
NGREK

SEQ ID NO: 30 - protein, 5 aa, synthetic construct
  REGION 1..5: note = circular
CNGRC